European Patent Specification EP 4 107 293 B1, published April 24, 2024. Title: BACTERIAL STRAIN AND MEDICAL USES THEREOF. Applicant: AILEENS PHARMA S.R.L. The sequence listing filed with the application follows.

SEQUENCE LISTING (10 sequences)

SEQ ID NO: 1 - DNA, 20 bp, Artificial Sequence
  EF1 Forward primer
aacctccttacagtgaatcc

SEQ ID NO: 2 - DNA, 18 bp, Artificial Sequence
  EF1 Reverse primer
atgttatctccgtgccag

SEQ ID NO: 3 - DNA, 21 bp, Artificial Sequence
  Impi forward primer
tagtaagcagtagcatagtcc

SEQ ID NO: 4 - DNA, 18 bp, Artificial Sequence
  Impi reverse primer
gccatcttcacagtagca

SEQ ID NO: 5 - DNA, 20 bp, Artificial Sequence
  Glutaraldehyde forward primer
ccacactgtgaggcaacatt

SEQ ID NO: 6 - DNA, 20 bp, Artificial Sequence
  Glutaraldehyde reverse primer
gtttgcttagcacggtcaca

SEQ ID NO: 7 - DNA, 20 bp, Artificial Sequence
  Cytokine forward primer
cgagctaaagacaggcgatt

SEQ ID NO: 8 - DNA, 20 bp, Artificial Sequence
  Cytokine reverse primer
tcacctgcggttgaatcata

SEQ ID NO: 9 - DNA, 20 bp, Artificial Sequence
  Phagoc forward primer
attgctagccaggttcagga

SEQ ID NO: 10 - DNA, 20 bp, Artificial Sequence
  Phagoc reverse primer
agctatttggcggaaactca